European Patent Application EP 4 438 627 A1, published October 2, 2024. Title: ANTI-TROP-2 ANTIBODY OR ANTIGEN-BINDING FRAGMENT THEREOF. Applicant: Chia Tai Tianqing Pharmaceutical Group Co., Ltd. The sequence listing filed with the application follows.

SEQUENCE LISTING (78 sequences)

SEQ ID NO: 1 - protein, 323 aa, Homo sapiens
MARGPGLAPPPLRLPLLLLVLAAVTGHTAAQDNCTCPTNKMTVCSPDGPGGRCQCRALGSGMAVDCSTLTSKCLLLKARMSAPKNARTLVRPSEHALVDNDGLYDPDCDPEGRFKARQCNQTSVCWCVNSVGVRRTDKGDLSLRCDELVRTHHILIDLRHRPTAGAFNHSDLDAELRRLFRERYRLHPKFVAAVHYEQPTIQIELRQNTSQKAAGDVDIGDAAYYFERDIKGESLFQGRGGLDLRVRGEPLQVERTLIYYLDEIPPKFSMKRLTAGLIAVIVVVVVALVAGMAVLVITNRRKSGKYKKVEIKELGELRKEPSL

SEQ ID NO: 2 - protein, 513 aa, synthetic construct
  source 1..513: note = Human TROP2-hFc
MARGPGLAPPPLRLPLLLLVLAAVTGHTAAQDNCTCPTNKMTVCSPDGPGGRCQCRALGSGMAVDCSTLTSKCLLLKARMSAPKNARTLVRPSEHALVDNDGLYDPDCDPEGRFKARQCNQTSVCWCVNSVGVRRTDKGDLSLRCDELVRTHHILIDLRHRPTAGAFNHSDLDAELRRLFRERYRLHPKFVAAVHYEQPTIQIELRQNTSQKAAGDVDIGDAAYYFERDIKGESLFQGRGGLDLRVRGEPLQVERTLIYYLDEIPPKFSMKRLTGGGSGGGSPKSSDKTHTCPPCPAPELLGGPSVFLFPPKPKDTLMISRTPEVTCVVVDVSHEDPEVKFNWYVDGVEVHNAKTKPREEQYNSTYRVVSVLTVLHQDWLNGKEYKCKVSNKALPAPIEKTISKAKGQPREPQVYTLPPSRDELTKNQVSLTCLVKGFYPSDIAVEWESNGQPENNYKTTPPVLDSDGSFFLYSKLTVDKSRWQQGNVFSCSVMHEALHNHYTQKSLSLSPGK

SEQ ID NO: 3 - protein, 292 aa, synthetic construct
  source 1..292: note = Human Trop-2-His
MARGPGLAPPPLRLPLLLLVLAAVTGHTAAQDNCTCPTNKMTVCSPDGPGGRCQCRALGSGMAVDCSTLTSKCLLLKARMSAPKNARTLVRPSEHALVDNDGLYDPDCDPEGRFKARQCNQTSVCWCVNSVGVRRTDKGDLSLRCDELVRTHHILIDLRHRPTAGAFNHSDLDAELRRLFRERYRLHPKFVAAVHYEQPTIQIELRQNTSQKAAGDVDIGDAAYYFERDIKGESLFQGRGGLDLRVRGEPLQVERTLIYYLDEIPPKFSMKRLTGGGSGGGSHHHHHHHHHH

SEQ ID NO: 4 - protein, 292 aa, synthetic construct
  source 1..292: note = Macaque Trop-2-His
MARGPGLAPPPLRLPLLLLLLAAVTGHTAAQDNCTCPTNKMTVCSPDGPGGRCQCRALGSGVAVDCSTLTSKCLLLKARMSAPKNARTLVRPNEHALVDNDGLYDPDCDPEGRFKARQCNQTSVCWCVNSVGVRRTDKGDLSLRCDELVRTHHILIDLRHRPTAGAFNHSDLDAELRRLFRERYRLHPKFVAAVHYEQPTIQIELRQNTSQKAAGDVDIGDAAYYFERDVKGESLFQGRGGLDLRVRGEPLQVERTLIYYLDEIPPKFSMKRLTGGGSGGGSHHHHHHHHHH

SEQ ID NO: 5 - protein, 10 aa, Mus musculus
GFSLTYYGID

SEQ ID NO: 6 - protein, 16 aa, Mus musculus
VIWGSGNTKYNSALMS

SEQ ID NO: 7 - protein, 7 aa, Mus musculus
FYEGFAY

SEQ ID NO: 8 - protein, 11 aa, Mus musculus
KASQDINSYLS

SEQ ID NO: 9 - protein, 7 aa, Mus musculus
RANRLVD

SEQ ID NO: 10 - protein, 9 aa, Mus musculus
LQYDEFPLT

SEQ ID NO: 11 - protein, 10 aa, Mus musculus
GFSLRNYGVH

SEQ ID NO: 12 - protein, 17 aa, Mus musculus
VIWSSGTTDYNAAFISR

SEQ ID NO: 13 - protein, 11 aa, Mus musculus
DGDYDYYTMDY

SEQ ID NO: 14 - protein, 15 aa, Mus musculus
RASKSVSTSAYSYIH

SEQ ID NO: 15 - protein, 7 aa, Mus musculus
LTSNLES

SEQ ID NO: 16 - protein, 9 aa, Mus musculus
QHSRELPYT

SEQ ID NO: 17 - protein, 10 aa, Mus musculus
GYTFTSSDIN

SEQ ID NO: 18 - protein, 17 aa, Mus musculus
WIYPRDGSKKYNEKFKG

SEQ ID NO: 19 - protein, 13 aa, Mus musculus
RFATVVSNYGLDP

SEQ ID NO: 20 - protein, 10 aa, Mus musculus
SASSSVNYIY

SEQ ID NO: 21 - protein, 7 aa, Mus musculus
DTSNLAS

SEQ ID NO: 22 - protein, 9 aa, Mus musculus
QQWNSYPLT

SEQ ID NO: 23 - protein, 115 aa, Mus musculus
EVQLVESGPGLVAPSQSLSITCTVSGFSLTYYGIDWVRQPPGKGLEWLGVIWGSGNTKYNSALMSRLSISKDNSKSQVFLRMNSLQSDDTAIYYCARFYEGFAYWGQGTLVTVSA

SEQ ID NO: 24 - protein, 107 aa, Mus musculus
AIVLTQSPSSMYASLGERVTITCKASQDINSYLSWFQQKPGKSPKTLIYRANRLVDGVPSRFSGSGSGQDYSLTISSLEYEDMGIYYCLQYDEFPLTFGVGTKLELK

SEQ ID NO: 25 - protein, 119 aa, Mus musculus
EVQLKQSGPGLVQPSQSLSITCTVSGFSLRNYGVHWVRQSPGKGLEWLGVIWSSGTTDYNAAFISRLSITKDNSKSQVFFKMNSLQVDDTAIYNCARDGDYDYYTMDYWGQGTSVTVSS

SEQ ID NO: 26 - protein, 111 aa, Mus musculus
AIVLTQSPASLAVSLGQRATISCRASKSVSTSAYSYIHWYQQKPGQPPKLLIYLTSNLESGVPARFSGSGSGTDFTLNIHPVEEEDAATYYCQHSRELPYTFGGGTKLEIK

SEQ ID NO: 27 - protein, 122 aa, Mus musculus
EVQLQQSGPDLVRPGASVKLSCKASGYTFTSSDINWVKQRPGQGLEWIGWIYPRDGSKKYNEKFKGKATLTVDTSSSTAYMEVHSLTSEDSAVYFCATRFATVVSNYGLDPWGQGTSVTVSS

SEQ ID NO: 28 - protein, 106 aa, Mus musculus
AIVLTQSPAIMSASPGEKVTMTCSASSSVNYIYWYQRKPGSSPRLLIYDTSNLASGVPVRFSGSGSGTSYSLTISRMEAEDAATYYCQQWNSYPLTFGAGTKLELK

SEQ ID NO: 29 - protein, 330 aa, Homo sapiens [sequence omitted]

SEQ ID NO: 30 - protein, 107 aa, Homo sapiens [sequence omitted]

SEQ ID NO: 31 - protein, 16 aa, synthetic construct
  source 1..16: note = Heavy chain CDR2
VIWGSGNTKYNSALKS

SEQ ID NO: 32 - protein, 16 aa, synthetic construct
  source 1..16: note = Heavy chain CDR2
VIWGSGNTKYNYALKS

SEQ ID NO: 33 - protein, 11 aa, synthetic construct
  source 1..11: note = Light chain CDR1
RASQDINSYLS

SEQ ID NO: 34 - protein, 7 aa, synthetic construct
  source 1..7: note = Light chain CDR2
RANRLVE

SEQ ID NO: 35 - protein, 9 aa, synthetic construct
  source 1..9: note = Light chain CDR3
LQYDEYPLT

SEQ ID NO: 36 - protein, 115 aa, synthetic construct
  source 1..115: note = Heavy chain variable region
EVQLVESGGGLIQPGGSLRLSCAVSGFSLTYYGIDWVRQPPGKGLEWVSVIWGSGNTKYNSALKSRLTISRDNSKSTLYLQMNSLRAEDTAVYYCARFYEGFAYWGQGTLVTVSS

SEQ ID NO: 37 - protein, 115 aa, synthetic construct
  source 1..115: note = Heavy chain variable region
EVQLVESGPGLIQPGGSLRLSCAVSGFSLTYYGIDWVRQPPGKGLEWVGVIWGSGNTKYNYALKSRLTISKDNSKSTLYLQMNSLRAEDTAVYYCARFYEGFAYWGQGTLVTVSS

SEQ ID NO: 38 - protein, 115 aa, synthetic construct
  source 1..115: note = Heavy chain variable region
QVQLQESGPGLVKPSETLSLTCTVSGFSLTYYGIDWIRQPPGKGLEWIGVIWGSGNTKYNSALKSRVTISKDNSKSQFSLKLSSVTAADTAVYYCARFYEGFAYWGQGTLVTVSS

SEQ ID NO: 39 - protein, 115 aa, synthetic construct
  source 1..115: note = Heavy chain variable region
QVQLQESGPGLVKPSETLSLTCTVSGFSLTYYGIDWIRQPPGKGLEWIGVIWGSGNTKYNSALKSRVTISKDNSKSQVYLKLSSVTAADTAVYYCARFYEGFAYWGQGTLVTVSS

SEQ ID NO: 40 - protein, 107 aa, synthetic construct
  source 1..107: note = Light chain variable region
DIQMTQSPSSLSASVGDRVTITCKASQDINSYLSWFQQKPGKAPKTLIYRANRLVEGVPSRFSGSGSGQDYTLTISSLQPEDFATYYCLQYDEFPLTFGQGTKVEIK

SEQ ID NO: 41 - protein, 107 aa, synthetic construct
  source 1..107: note = Light chain variable region
DIQMTQSPSSLSASVGDRVTITCRASQDINSYLSWFQQKPGKAPKTLIYRANRLVEGVPSRFSGSGSGQDFTLTISSLQPEDFATYYCLQYDEYPLTFGQGTKVEIK

SEQ ID NO: 42 - protein, 445 aa, synthetic construct
  source 1..445: note = Heavy chain
EVQLVESGGGLIQPGGSLRLSCAVSGFSLTYYGIDWVRQPPGKGLEWVSVIWGSGNTKYNSALKSRLTISRDNSKSTLYLQMNSLRAEDTAVYYCARFYEGFAYWGQGTLVTVSSASTKGPSVFPLAPSSKSTSGGTAALGCLVKDYFPEPVTVSWNSGALTSGVHTFPAVLQSSGLYSLSSVVTVPSSSLGTQTYICNVNHKPSNTKVDKKVEPKSCDKTHTCPPCPAPELLGGPSVFLFPPKPKDTLMISRTPEVTCVVVDVSHEDPEVKFNWYVDGVEVHNAKTKPREEQYNSTYRVVSVLTVLHQDWLNGKEYKCKVSNKALPAPIEKTISKAKGQPREPQVYTLPPSRDELTKNQVSLTCLVKGFYPSDIAVEWESNGQPENNYKTTPPVLDSDGSFFLYSKLTVDKSRWQQGNVFSCSVMHEALHNHYTQKSLSLSPGK

SEQ ID NO: 43 - protein, 445 aa, synthetic construct
  source 1..445: note = Heavy chain
EVQLVESGPGLIQPGGSLRLSCAVSGFSLTYYGIDWVRQPPGKGLEWVGVIWGSGNTKYNYALKSRLTISKDNSKSTLYLQMNSLRAEDTAVYYCARFYEGFAYWGQGTLVTVSSASTKGPSVFPLAPSSKSTSGGTAALGCLVKDYFPEPVTVSWNSGALTSGVHTFPAVLQSSGLYSLSSVVTVPSSSLGTQTYICNVNHKPSNTKVDKKVEPKSCDKTHTCPPCPAPELLGGPSVFLFPPKPKDTLMISRTPEVTCVVVDVSHEDPEVKFNWYVDGVEVHNAKTKPREEQYNSTYRVVSVLTVLHQDWLNGKEYKCKVSNKALPAPIEKTISKAKGQPREPQVYTLPPSRDELTKNQVSLTCLVKGFYPSDIAVEWESNGQPENNYKTTPPVLDSDGSFFLYSKLTVDKSRWQQGNVFSCSVMHEALHNHYTQKSLSLSPGK

SEQ ID NO: 44 - protein, 445 aa, synthetic construct
  source 1..445: note = Heavy chain
QVQLQESGPGLVKPSETLSLTCTVSGFSLTYYGIDWIRQPPGKGLEWIGVIWGSGNTKYNSALKSRVTISKDNSKSQFSLKLSSVTAADTAVYYCARFYEGFAYWGQGTLVTVSSASTKGPSVFPLAPSSKSTSGGTAALGCLVKDYFPEPVTVSWNSGALTSGVHTFPAVLQSSGLYSLSSVVTVPSSSLGTQTYICNVNHKPSNTKVDKKVEPKSCDKTHTCPPCPAPELLGGPSVFLFPPKPKDTLMISRTPEVTCVVVDVSHEDPEVKFNWYVDGVEVHNAKTKPREEQYNSTYRVVSVLTVLHQDWLNGKEYKCKVSNKALPAPIEKTISKAKGQPREPQVYTLPPSRDELTKNQVSLTCLVKGFYPSDIAVEWESNGQPENNYKTTPPVLDSDGSFFLYSKLTVDKSRWQQGNVFSCSVMHEALHNHYTQKSLSLSPGK

SEQ ID NO: 45 - protein, 445 aa, synthetic construct
  source 1..445: note = Heavy chain
QVQLQESGPGLVKPSETLSLTCTVSGFSLTYYGIDWIRQPPGKGLEWIGVIWGSGNTKYNSALKSRVTISKDNSKSQVYLKLSSVTAADTAVYYCARFYEGFAYWGQGTLVTVSSASTKGPSVFPLAPSSKSTSGGTAALGCLVKDYFPEPVTVSWNSGALTSGVHTFPAVLQSSGLYSLSSVVTVPSSSLGTQTYICNVNHKPSNTKVDKKVEPKSCDKTHTCPPCPAPELLGGPSVFLFPPKPKDTLMISRTPEVTCVVVDVSHEDPEVKFNWYVDGVEVHNAKTKPREEQYNSTYRVVSVLTVLHQDWLNGKEYKCKVSNKALPAPIEKTISKAKGQPREPQVYTLPPSRDELTKNQVSLTCLVKGFYPSDIAVEWESNGQPENNYKTTPPVLDSDGSFFLYSKLTVDKSRWQQGNVFSCSVMHEALHNHYTQKSLSLSPGK

SEQ ID NO: 46 - protein, 214 aa, synthetic construct
  source 1..214: note = Light chain
DIQMTQSPSSLSASVGDRVTITCKASQDINSYLSWFQQKPGKAPKTLIYRANRLVEGVPSRFSGSGSGQDYTLTISSLQPEDFATYYCLQYDEFPLTFGQGTKVEIKRTVAAPSVFIFPPSDEQLKSGTASVVCLLNNFYPREAKVQWKVDNALQSGNSQESVTEQDSKDSTYSLSSTLTLSKADYEKHKVYACEVTHQGLSSPVTKSFNRGEC

SEQ ID NO: 47 - protein, 214 aa, synthetic construct
  source 1..214: note = Light chain
DIQMTQSPSSLSASVGDRVTITCRASQDINSYLSWFQQKPGKAPKTLIYRANRLVEGVPSRFSGSGSGQDFTLTISSLQPEDFATYYCLQYDEYPLTFGQGTKVEIKRTVAAPSVFIFPPSDEQLKSGTASVVCLLNNFYPREAKVQWKVDNALQSGNSQESVTEQDSKDSTYSLSSTLTLSKADYEKHKVYACEVTHQGLSSPVTKSFNRGEC

SEQ ID NO: 48 - protein, 10 aa, synthetic construct
  source 1..10: note = Heavy chain CDR1
GFTLRNYGVH

SEQ ID NO: 49 - protein, 16 aa, synthetic construct
  source 1..16: note = Heavy chain CDR2
VIWSSGTTDYAAPVKG

SEQ ID NO: 50 - protein, 119 aa, synthetic construct
  source 1..119: note = Heavy chain variable region
EVQLVESGGGLVKPGGSLRLSCAASGFTLRNYGVHWVRQAPGKGLEWVGVIWSSGTTDYAAPVKGRFTISKDNSKNTLYLQMNSLKTEDTAVYYCTRDGDYDYYTMDYWGQGTLVTVSS

SEQ ID NO: 51 - protein, 119 aa, synthetic construct
  source 1..119: note = Heavy chain variable region
EVQLVESGGGLVKPGGSLRLSCAASGFTLRNYGVHWVRQAPGKGLEWVGVIWSSGTTDYNAAFISRFTISKDNSKNTLYLQMNSLKTEDTAVYYCTRDGDYDYYTMDYWGQGTLVTVSS

SEQ ID NO: 52 - protein, 119 aa, synthetic construct
  source 1..119: note = Heavy chain variable region
EVQLVESGGGLVKPGGSLRLSCAASGFTLRNYGVHWVRQAPGKGLEWVGVIWSSGTTDYAAPVKGRFTISKDNSKNTLYLQMNSLKTEDTAVYNCTRDGDYDYYTMDYWGQGTLVTVSS

SEQ ID NO: 53 - protein, 119 aa, synthetic construct
  source 1..119: note = Heavy chain variable region
EVQLVESGGGLVKPGGSLRLSCAASGFTLRNYGVHWVRQAPGKGLEWVGVIWSSGTTDYNAAFISRFTISKDNSKNTLYLQMNSLKTEDTAVYNCTRDGDYDYYTMDYWGQGTLVTVSS

SEQ ID NO: 54 - protein, 111 aa, synthetic construct
  source 1..111: note = Light chain variable region
EIVLTQSPATLSLSPGERATLSCRASKSVSTSAYSYIHWYQQKPGQAPRLLIYLTSNLESGIPARFSGSGSGTDFTLTISSLEPEDFAVYYCQHSRELPYTFGQGTKVEIK

SEQ ID NO: 55 - protein, 111 aa, synthetic construct
  source 1..111: note = Light chain variable region
EIVLTQSPATLSLSPGERATLSCRASKSVSTSAYSYIHWYQQKPGQPPRLLIYLTSNLESGIPARFSGSGSGTDFTLTISSLEPEDFAVYYCQHSRELPYTFGQGTKVEIK

SEQ ID NO: 56 - protein, 449 aa, synthetic construct
  source 1..449: note = Heavy chain
EVQLVESGGGLVKPGGSLRLSCAASGFTLRNYGVHWVRQAPGKGLEWVGVIWSSGTTDYAAPVKGRFTISKDNSKNTLYLQMNSLKTEDTAVYYCTRDGDYDYYTMDYWGQGTLVTVSSASTKGPSVFPLAPSSKSTSGGTAALGCLVKDYFPEPVTVSWNSGALTSGVHTFPAVLQSSGLYSLSSVVTVPSSSLGTQTYICNVNHKPSNTKVDKKVEPKSCDKTHTCPPCPAPELLGGPSVFLFPPKPKDTLMISRTPEVTCVVVDVSHEDPEVKFNWYVDGVEVHNAKTKPREEQYNSTYRVVSVLTVLHQDWLNGKEYKCKVSNKALPAPIEKTISKAKGQPREPQVYTLPPSRDELTKNQVSLTCLVKGFYPSDIAVEWESNGQPENNYKTTPPVLDSDGSFFLYSKLTVDKSRWQQGNVFSCSVMHEALHNHYTQKSLSLSPGK

SEQ ID NO: 57 - protein, 449 aa, synthetic construct
  source 1..449: note = Heavy chain
EVQLVESGGGLVKPGGSLRLSCAASGFTLRNYGVHWVRQAPGKGLEWVGVIWSSGTTDYNAAFISRFTISKDNSKNTLYLQMNSLKTEDTAVYYCTRDGDYDYYTMDYWGQGTLVTVSSASTKGPSVFPLAPSSKSTSGGTAALGCLVKDYFPEPVTVSWNSGALTSGVHTFPAVLQSSGLYSLSSVVTVPSSSLGTQTYICNVNHKPSNTKVDKKVEPKSCDKTHTCPPCPAPELLGGPSVFLFPPKPKDTLMISRTPEVTCVVVDVSHEDPEVKFNWYVDGVEVHNAKTKPREEQYNSTYRVVSVLTVLHQDWLNGKEYKCKVSNKALPAPIEKTISKAKGQPREPQVYTLPPSRDELTKNQVSLTCLVKGFYPSDIAVEWESNGQPENNYKTTPPVLDSDGSFFLYSKLTVDKSRWQQGNVFSCSVMHEALHNHYTQKSLSLSPGK

SEQ ID NO: 58 - protein, 449 aa, synthetic construct
  source 1..449: note = Heavy chain
EVQLVESGGGLVKPGGSLRLSCAASGFTLRNYGVHWVRQAPGKGLEWVGVIWSSGTTDYAAPVKGRFTISKDNSKNTLYLQMNSLKTEDTAVYNCTRDGDYDYYTMDYWGQGTLVTVSSASTKGPSVFPLAPSSKSTSGGTAALGCLVKDYFPEPVTVSWNSGALTSGVHTFPAVLQSSGLYSLSSVVTVPSSSLGTQTYICNVNHKPSNTKVDKKVEPKSCDKTHTCPPCPAPELLGGPSVFLFPPKPKDTLMISRTPEVTCVVVDVSHEDPEVKFNWYVDGVEVHNAKTKPREEQYNSTYRVVSVLTVLHQDWLNGKEYKCKVSNKALPAPIEKTISKAKGQPREPQVYTLPPSRDELTKNQVSLTCLVKGFYPSDIAVEWESNGQPENNYKTTPPVLDSDGSFFLYSKLTVDKSRWQQGNVFSCSVMHEALHNHYTQKSLSLSPGK

SEQ ID NO: 59 - protein, 449 aa, synthetic construct
  source 1..449: note = Heavy chain
EVQLVESGGGLVKPGGSLRLSCAASGFTLRNYGVHWVRQAPGKGLEWVGVIWSSGTTDYNAAFISRFTISKDNSKNTLYLQMNSLKTEDTAVYNCTRDGDYDYYTMDYWGQGTLVTVSSASTKGPSVFPLAPSSKSTSGGTAALGCLVKDYFPEPVTVSWNSGALTSGVHTFPAVLQSSGLYSLSSVVTVPSSSLGTQTYICNVNHKPSNTKVDKKVEPKSCDKTHTCPPCPAPELLGGPSVFLFPPKPKDTLMISRTPEVTCVVVDVSHEDPEVKFNWYVDGVEVHNAKTKPREEQYNSTYRVVSVLTVLHQDWLNGKEYKCKVSNKALPAPIEKTISKAKGQPREPQVYTLPPSRDELTKNQVSLTCLVKGFYPSDIAVEWESNGQPENNYKTTPPVLDSDGSFFLYSKLTVDKSRWQQGNVFSCSVMHEALHNHYTQKSLSLSPGK

SEQ ID NO: 60 - protein, 218 aa, synthetic construct
  source 1..218: note = Light chain
EIVLTQSPATLSLSPGERATLSCRASKSVSTSAYSYIHWYQQKPGQAPRLLIYLTSNLESGIPARFSGSGSGTDFTLTISSLEPEDFAVYYCQHSRELPYTFGQGTKVEIKRTVAAPSVFIFPPSDEQLKSGTASVVCLLNNFYPREAKVQWKVDNALQSGNSQESVTEQDSKDSTYSLSSTLTLSKADYEKHKVYACEVTHQGLSSPVTKSFNRGEC

SEQ ID NO: 61 - protein, 218 aa, synthetic construct
  source 1..218: note = Light chain
EIVLTQSPATLSLSPGERATLSCRASKSVSTSAYSYIHWYQQKPGQPPRLLIYLTSNLESGIPARFSGSGSGTDFTLTISSLEPEDFAVYYCQHSRELPYTFGQGTKVEIKRTVAAPSVFIFPPSDEQLKSGTASVVCLLNNFYPREAKVQWKVDNALQSGNSQESVTEQDSKDSTYSLSSTLTLSKADYEKHKVYACEVTHQGLSSPVTKSFNRGEC

SEQ ID NO: 62 - protein, 17 aa, synthetic construct
  source 1..17: note = Heavy chain CDR2
WIYPRDGSKKYAQKFQG

SEQ ID NO: 63 - protein, 122 aa, synthetic construct
  source 1..122: note = Heavy chain variable region
QVQLVQSGAEVKKPGASVKVSCKASGYTFTSSDINWVRQRPGQGLEWMGWIYPRDGSKKYAQKFQGRVTMTVDTSTSTVYMELSSLRSEDTAVYYCATRFATVVSNYGLDPWGQGTLVTVSS

SEQ ID NO: 64 - protein, 122 aa, synthetic construct
  source 1..122: note = Heavy chain variable region
QVQLVQSGAEVKKPGASVKVSCKASGYTFTSSDINWVRQRPGQGLEWMGWIYPRDGSKKYNEKFKGRVTMTVDTSTSTVYMELSSLRSEDTAVYYCARRFATVVSNYGLDPWGQGTLVTVSS

SEQ ID NO: 65 - protein, 122 aa, synthetic construct
  source 1..122: note = Heavy chain variable region
QVQLVQSGAEVKKPGASVKVSCKASGYTFTSSDINWVRQRPGQGLEWMGWIYPRDGSKKYNEKFKGRVTMTVDTSTSTVYMELSSLRSEDTAVYYCATRFATVVSNYGLDPWGQGTLVTVSS

SEQ ID NO: 66 - protein, 106 aa, synthetic construct
  source 1..106: note = Light chain variable region
EIVLTQSPATLSLSPGERATLSCSASSSVNYIYWYQRKPGQAPRLLIYDTSNLASGIPARFSGSGSGTDFTLTISSLEPEDFAVYYCQQWNSYPLTFGQGTKVEIK

SEQ ID NO: 67 - protein, 106 aa, synthetic construct
  source 1..106: note = Light chain variable region
EIVLTQSPATLSLSPGERATLSCSASSSVNYIYWYQRKPGQAPRLLIYDTSNLASGIPARFSGSGSGTDYTLTISSLEPEDFAVYYCQQWNSYPLTFGQGTKVEIK

SEQ ID NO: 68 - protein, 452 aa, synthetic construct
  source 1..452: note = Heavy chain
QVQLVQSGAEVKKPGASVKVSCKASGYTFTSSDINWVRQRPGQGLEWMGWIYPRDGSKKYAQKFQGRVTMTVDTSTSTVYMELSSLRSEDTAVYYCATRFATVVSNYGLDPWGQGTLVTVSSASTKGPSVFPLAPSSKSTSGGTAALGCLVKDYFPEPVTVSWNSGALTSGVHTFPAVLQSSGLYSLSSVVTVPSSSLGTQTYICNVNHKPSNTKVDKKVEPKSCDKTHTCPPCPAPELLGGPSVFLFPPKPKDTLMISRTPEVTCVVVDVSHEDPEVKFNWYVDGVEVHNAKTKPREEQYNSTYRVVSVLTVLHQDWLNGKEYKCKVSNKALPAPIEKTISKAKGQPREPQVYTLPPSRDELTKNQVSLTCLVKGFYPSDIAVEWESNGQPENNYKTTPPVLDSDGSFFLYSKLTVDKSRWQQGNVFSCSVMHEALHNHYTQKSLSLSPGK

SEQ ID NO: 69 - protein, 452 aa, synthetic construct
  source 1..452: note = Heavy chain
QVQLVQSGAEVKKPGASVKVSCKASGYTFTSSDINWVRQRPGQGLEWMGWIYPRDGSKKYNEKFKGRVTMTVDTSTSTVYMELSSLRSEDTAVYYCARRFATVVSNYGLDPWGQGTLVTVSSASTKGPSVFPLAPSSKSTSGGTAALGCLVKDYFPEPVTVSWNSGALTSGVHTFPAVLQSSGLYSLSSVVTVPSSSLGTQTYICNVNHKPSNTKVDKKVEPKSCDKTHTCPPCPAPELLGGPSVFLFPPKPKDTLMISRTPEVTCVVVDVSHEDPEVKFNWYVDGVEVHNAKTKPREEQYNSTYRVVSVLTVLHQDWLNGKEYKCKVSNKALPAPIEKTISKAKGQPREPQVYTLPPSRDELTKNQVSLTCLVKGFYPSDIAVEWESNGQPENNYKTTPPVLDSDGSFFLYSKLTVDKSRWQQGNVFSCSVMHEALHNHYTQKSLSLSPGK

SEQ ID NO: 70 - protein, 452 aa, synthetic construct
  source 1..452: note = Heavy chain
QVQLVQSGAEVKKPGASVKVSCKASGYTFTSSDINWVRQRPGQGLEWMGWIYPRDGSKKYNEKFKGRVTMTVDTSTSTVYMELSSLRSEDTAVYYCATRFATVVSNYGLDPWGQGTLVTVSSASTKGPSVFPLAPSSKSTSGGTAALGCLVKDYFPEPVTVSWNSGALTSGVHTFPAVLQSSGLYSLSSVVTVPSSSLGTQTYICNVNHKPSNTKVDKKVEPKSCDKTHTCPPCPAPELLGGPSVFLFPPKPKDTLMISRTPEVTCVVVDVSHEDPEVKFNWYVDGVEVHNAKTKPREEQYNSTYRVVSVLTVLHQDWLNGKEYKCKVSNKALPAPIEKTISKAKGQPREPQVYTLPPSRDELTKNQVSLTCLVKGFYPSDIAVEWESNGQPENNYKTTPPVLDSDGSFFLYSKLTVDKSRWQQGNVFSCSVMHEALHNHYTQKSLSLSPGK

SEQ ID NO: 71 - protein, 213 aa, synthetic construct
  source 1..213: note = Light chain
EIVLTQSPATLSLSPGERATLSCSASSSVNYIYWYQRKPGQAPRLLIYDTSNLASGIPARFSGSGSGTDFTLTISSLEPEDFAVYYCQQWNSYPLTFGQGTKVEIKRTVAAPSVFIFPPSDEQLKSGTASVVCLLNNFYPREAKVQWKVDNALQSGNSQESVTEQDSKDSTYSLSSTLTLSKADYEKHKVYACEVTHQGLSSPVTKSFNRGEC

SEQ ID NO: 72 - protein, 213 aa, synthetic construct
  source 1..213: note = Light chain
EIVLTQSPATLSLSPGERATLSCSASSSVNYIYWYQRKPGQAPRLLIYDTSNLASGIPARFSGSGSGTDYTLTISSLEPEDFAVYYCQQWNSYPLTFGQGTKVEIKRTVAAPSVFIFPPSDEQLKSGTASVVCLLNNFYPREAKVQWKVDNALQSGNSQESVTEQDSKDSTYSLSSTLTLSKADYEKHKVYACEVTHQGLSSPVTKSFNRGEC

SEQ ID NO: 73 - protein, 445 aa, synthetic construct
  source 1..445: note = Chimeric heavy chain of ch-Ab2
EVQLVESGPGLVAPSQSLSITCTVSGFSLTYYGIDWVRQPPGKGLEWLGVIWGSGNTKYNSALMSRLSISKDNSKSQVFLRMNSLQSDDTAIYYCARFYEGFAYWGQGTLVTVSAASTKGPSVFPLAPSSKSTSGGTAALGCLVKDYFPEPVTVSWNSGALTSGVHTFPAVLQSSGLYSLSSVVTVPSSSLGTQTYICNVNHKPSNTKVDKKVEPKSCDKTHTCPPCPAPELLGGPSVFLFPPKPKDTLMISRTPEVTCVVVDVSHEDPEVKFNWYVDGVEVHNAKTKPREEQYNSTYRVVSVLTVLHQDWLNGKEYKCKVSNKALPAPIEKTISKAKGQPREPQVYTLPPSRDELTKNQVSLTCLVKGFYPSDIAVEWESNGQPENNYKTTPPVLDSDGSFFLYSKLTVDKSRWQQGNVFSCSVMHEALHNHYTQKSLSLSPGK

SEQ ID NO: 74 - protein, 214 aa, synthetic construct
  source 1..214: note = Chimeric light chain of ch-Ab2
AIVLTQSPSSMYASLGERVTITCKASQDINSYLSWFQQKPGKSPKTLIYRANRLVDGVPSRFSGSGSGQDYSLTISSLEYEDMGIYYCLQYDEFPLTFGVGTKLELKRTVAAPSVFIFPPSDEQLKSGTASVVCLLNNFYPREAKVQWKVDNALQSGNSQESVTEQDSKDSTYSLSSTLTLSKADYEKHKVYACEVTHQGLSSPVTKSFNRGEC

SEQ ID NO: 75 - protein, 449 aa, synthetic construct
  source 1..449: note = Chimeric heavy chain of ch-Ab21
EVQLKQSGPGLVQPSQSLSITCTVSGFSLRNYGVHWVRQSPGKGLEWLGVIWSSGTTDYNAAFISRLSITKDNSKSQVFFKMNSLQVDDTAIYNCARDGDYDYYTMDYWGQGTSVTVSSASTKGPSVFPLAPSSKSTSGGTAALGCLVKDYFPEPVTVSWNSGALTSGVHTFPAVLQSSGLYSLSSVVTVPSSSLGTQTYICNVNHKPSNTKVDKKVEPKSCDKTHTCPPCPAPELLGGPSVFLFPPKPKDTLMISRTPEVTCVVVDVSHEDPEVKFNWYVDGVEVHNAKTKPREEQYNSTYRVVSVLTVLHQDWLNGKEYKCKVSNKALPAPIEKTISKAKGQPREPQVYTLPPSRDELTKNQVSLTCLVKGFYPSDIAVEWESNGQPENNYKTTPPVLDSDGSFFLYSKLTVDKSRWQQGNVFSCSVMHEALHNHYTQKSLSLSPGK

SEQ ID NO: 76 - protein, 218 aa, synthetic construct
  source 1..218: note = Chimeric light chain of ch-Ab21
AIVLTQSPASLAVSLGQRATISCRASKSVSTSAYSYIHWYQQKPGQPPKLLIYLTSNLESGVPARFSGSGSGTDFTLNIHPVEEEDAATYYCQHSRELPYTFGGGTKLEIKRTVAAPSVFIFPPSDEQLKSGTASVVCLLNNFYPREAKVQWKVDNALQSGNSQESVTEQDSKDSTYSLSSTLTLSKADYEKHKVYACEVTHQGLSSPVTKSFNRGEC

SEQ ID NO: 77 - protein, 452 aa, synthetic construct
  source 1..452: note = Chimeric heavy chain of ch-Ab35
EVQLQQSGPDLVRPGASVKLSCKASGYTFTSSDINWVKQRPGQGLEWIGWIYPRDGSKKYNEKFKGKATLTVDTSSSTAYMEVHSLTSEDSAVYFCATRFATVVSNYGLDPWGQGTSVTVSSASTKGPSVFPLAPSSKSTSGGTAALGCLVKDYFPEPVTVSWNSGALTSGVHTFPAVLQSSGLYSLSSVVTVPSSSLGTQTYICNVNHKPSNTKVDKKVEPKSCDKTHTCPPCPAPELLGGPSVFLFPPKPKDTLMISRTPEVTCVVVDVSHEDPEVKFNWYVDGVEVHNAKTKPREEQYNSTYRVVSVLTVLHQDWLNGKEYKCKVSNKALPAPIEKTISKAKGQPREPQVYTLPPSRDELTKNQVSLTCLVKGFYPSDIAVEWESNGQPENNYKTTPPVLDSDGSFFLYSKLTVDKSRWQQGNVFSCSVMHEALHNHYTQKSLSLSPGK

SEQ ID NO: 78 - protein, 213 aa, synthetic construct
  source 1..213: note = Chimeric light chain of ch-Ab35
AIVLTQSPAIMSASPGEKVTMTCSASSSVNYIYWYQRKPGSSPRLLIYDTSNLASGVPVRFSGSGSGTSYSLTISRMEAEDAATYYCQQWNSYPLTFGAGTKLELKRTVAAPSVFIFPPSDEQLKSGTASVVCLLNNFYPREAKVQWKVDNALQSGNSQESVTEQDSKDSTYSLSSTLTLSKADYEKHKVYACEVTHQGLSSPVTKSFNRGEC